European Patent Application EP 4 775 689 A2, published July 15, 2026. Title: SINGLE-CHANNEL SEQUENCING METHOD BASED ON SELF-LUMINESCENCE. Applicant: QINGDAO MGI TECH CO., LTD. The sequence listing filed with the application follows.

SEQUENCE LISTING (7 sequences)

SEQ ID NO: 1 - DNA, 233 bp, synthetic construct
  source 1..233: mol_type = other DNA; note = DNA sequence designed
gatatctgcaggcatagaatgaatattattgaatcaataattaaagtcggaggccaagcggtcttaggaagacaacaactccttggctcacagaacgacatggctacgatccgactttacaactacgataatgggctggatacatggaatgattatagatatattaaggaataatgttaattaatgcctaaattaattaatctaagggggttaatacttcagcctgtgatatc

SEQ ID NO: 2 - DNA, 15 bp, synthetic construct
  source 1..15: mol_type = other DNA; note = primer
gatatctgcaggcat

SEQ ID NO: 3 - DNA, 15 bp, synthetic construct
  source 1..15: mol_type = other DNA; note = primer
gatatcacaggctga

SEQ ID NO: 4 - DNA, 30 bp, synthetic construct
  source 1..30: mol_type = other DNA; note = split oligo
atgcctgcagatatcgatatcacaggctga

SEQ ID NO: 5 - DNA, 24 bp, synthetic construct
  source 1..24: mol_type = other DNA; note = primer
gccatgtcgttctgtgagccaagg

SEQ ID NO: 6 - DNA, 32 bp, synthetic construct
  source 1..32: mol_type = other DNA; note = primer
gctcacagaacgacatggctacgatccgactt

SEQ ID NO: 7 - DNA, 10 bp, synthetic construct
  source 1..10: mol_type = other DNA; note = the first 10bp base sequence
tacaactacg